European Patent Application EP 4 169 535 A1, published April 26, 2023. Title: METHODS AND COMPOSITIONS FOR DUAL GLYCAN BINDING AAV2.5 VECTOR. Applicant: The University of North Carolina at Chapel Hill. Application EP. The sequence listing filed with the application follows.

SEQUENCE LISTING (6 sequences)

SEQ ID NO: 1 - protein, 736 aa, synthetic construct
  REGION 1..736: note = AAV2.5 capsid protein
MAADGYLPDWLEDTLSEGIRQWWKLKPGPPPPKPAERHKDDSRGLVLPGYKYLGPFNGLDKGEPVNEADAAALEHDKAYDRQLDSGDNPYLKYNHADAEFQERLKEDTSFGGNLGRAVFQAKKRVLEPLGLVEEPVKTAPGKKRPVEHSPVEPDSSSGTGKAGQQPARKRLNFGQTGDADSVPDPQPLGQPPAAPSGLGTNTMATGSGAPMADNNEGADGVGNSSGNWHCDSTWMGDRVITTSTRTWALPTYNNHLYKQISSASTGASNDNHYFGYSTPWGYFDFNRFHCHFSPRDWQRLINNNWGFRPKRLNFKLFNIQVKEVTQNDGTTTIANNLTSTVQVFTDSEYQLPYVLGSAHQGCLPPFPADVFMVPQYGYLTLNNGSQAVGRSSFYCLEYFPSQMLRTGNNFTFSYTFEDVPFHSSYAHSQSLDRLMNPLIDQYLYYLSRTNTPSGTTTQSRLQFSQAGASDIRDQSRNWLPGPCYRQQRVSKTSADNNNSEYSWTGATKYHLNGRDSLVNPGPAMASHKDDEEKFFPQSGVLIFGKQGSEKTNVDIEKVMITDEEEIRTTNPVATEQYGSVSTNLQRGNRQAATADVNTQGVLPGMVWQDRDVYLQGPIWAKIPHTDGHFHPSPLMGGFGLKHPPPQILIKNTPVPANPSTTFSAAKFASFITQYSTGQVSVEIEWELQKENSKRWNPEIQYTSNYAKSANVDFTVDNNGVYSEPRPIGTRYLTRNL

SEQ ID NO: 2 - protein, 736 aa, synthetic construct
  REGION 1..736: note = AAV2.5G9 capsid protein
MAADGYLPDWLEDTLSEGIRQWWKLKPGPPPPKPAERHKDDSRGLVLPGYKYLGPFNGLDKGEPVNEADAAALEHDKAYDRQLDSGDNPYLKYNHADAEFQERLKEDTSFGGNLGRAVFQAKKRVLEPLGLVEEPVKTAPGKKRPVEHSPVEPDSSSGTGKAGQQPARKRLNFGQTGDADSVPDPQPLGQPPAAPSGLGTNTMATGSGAPMADNNEGADGVGNSSGNWHCDSTWMGDRVITTSTRTWALPTYNNHLYKQISSASTGSSNDNHYFGYSTPWGYFDFNRFHCHFSPRDWQRLINNNWGFRPKRLNFKLFNIQVKEVTQNDGTTTIANNLTSTVQVFTDSEYQLPYVLGSAHQGCLPPFPADVFMVPQYGYLTLNNGSQAVGRSSFYCLEYFPSQMLRTGNNFTFSYTFEDVPFHSSYAHSQSLDRLMNPLIDQYLYYLSRTNTPSGTTTQSRLQFSVAGPSNMAVQGRNWLPGPCYRQQRVSKTSADNNNSEFAWTGATKYHLNGRDSLVNPGPAMASHKDDEEKFFPQSGVLIFGKQGSEKTNVDIEKVMITDEEEIRTTNPVATEQYGSVSTNLQRGNRQAATADVNTQGVLPGMVWQDRDVYLQGPIWAKIPHTDGHFHPSPLMGGFGLKHPPPQILIKNTPVPANPSTTFSAAKFASFITQYSTGQVSVEIEWELQKENSKRWNPEIQYTSNYAKSANVDFTVDNNGVYSEPRPIGTRYLTRNL

SEQ ID NO: 3 - protein, 13 aa, adeno-associated virus 2.5
SQAGASDIRDQSR

SEQ ID NO: 4 - protein, 13 aa, synthetic construct
  REGION 1..13: note = AAV amino acid substitution sequence
  SITE 2: note = MISC_FEATURE - X is any amino acid as per defined in ST25 sequence listing standard
  SITE 5: note = MISC_FEATURE - X is any amino acid as per defined in ST25 sequence listing standard
  REGION 7..10: note = MISC_FEATURE - X is any amino acid as per defined in ST25 sequence listing standard
  SITE 12: note = MISC_FEATURE - X is any amino acid as per defined in ST25 sequence listing standard
SXAGXSXXXXQXR

SEQ ID NO: 5 - protein, 4 aa, adeno-associated virus 2.5
EYSW

SEQ ID NO: 6 - skipped